European Patent Application EP 4 434 349 A1, published September 25, 2024. Title: METHOD FOR OBTAINING Β-CASEIN. Applicant: Société des Produits Nestlé S.A. The sequence listing filed with the application follows.

SEQUENCE LISTING (1 sequence)

SEQ ID NO: 1 - protein, 381 aa, Camelus dromedarius
MRCLVVLLAALALSQASGITRIPLHKGKTLRKALKERGLLEDFLQRQQYAVSSKYSSLGKVAREPLTSYLDSQYFGKIYIGTPPQEFTVVFDTGSSDLWVPSIYCKSNVCKNHHRFDPRKSSTFRNLGKPLSIHYGTGSMEGFLGYDTVTVSNIVDPNQTVGLSTEQPGEVFTYSEFDGILGLAYPSLASEYSVPVFDNMMDRHLVARDLFSVYMDRNGQGSMLTLGAIDPSYYTGSLHWVPVTLQQYWQFTVDSVTINGVAVACVGGCQAILDTGTSVLFGPSSDILKIQMAIGATENRYGEFDVNCGNLRSMPTVVFEINGRDYPLSPSAYTSKDQGFCTSGFQGDNNSELWILGDVFIREYYSVFDRANNRVGLAKAI